European Patent Specification EP 4 356 135 B1, published December 10, 2025. Title: Thermostable Affinity Polypeptides. Applicant: Roche Diagnostics GmbH F. Hoffmann-La Roche AG Roche Diagnostics Operations, Inc. The sequence listing filed with the application follows.

SEQUENCE LISTING (19 sequences)

SEQ ID NO: 1 - protein, 115 aa, Geobacillus thermoglucosidasius
YNKGAIGIIPKEIRDKLVGKKFNSFDDFRKEFWKCVANSSYAKEFRSRNIARMLEGNAPIAPKAEHYGKLKSYILHHKQPIEKGGEVYNLDNLIITSPRMHQIILDPAYYFGKKG

SEQ ID NO: 2 - protein, 69 aa, Geobacillus thermoglucosidasius
ENKLSKEELIELVKKICDPKLSDEEVSEYIDILEKNVPHPAPSDLIFWNDEELSPEEIVEIALNYKDRN

SEQ ID NO: 3 - protein, 115 aa, Artificial Sequence
  Gth colicin polypeptide mutein fragment
YNKGAIGIIPKEIRDKLVGKKFNSFDDFRKEFWKAVANSSYAKEFRSRNIARMLEGNAPIAPKAEHYGKLKSYILHAKQPIEKGGEVYNLDNLIITSPRMHQIILDPAYYFGKKG

SEQ ID NO: 4 - protein, 69 aa, Artificial Sequence
  Gth immunity polypeptide mutein fragment
ENKLSKEELIELVKKIADPKLSDEEVSEYIDILEKNVPHPAPSDLIFWNDEELSPEEIVEIALNYKDRN

SEQ ID NO: 5 - protein, 6 aa, Artificial Sequence
  (His)6-tag
HHHHHH

SEQ ID NO: 6 - protein, 8 aa, Artificial Sequence
  (His)8-tag
HHHHHHHH

SEQ ID NO: 7 - protein, 4 aa, Artificial Sequence
  GGGS-linker
GGGS

SEQ ID NO: 8 - protein, 20 aa, Artificial Sequence
  (GGGS)5-Linker
GGGSGGGSGGGSGGGSGGGS

SEQ ID NO: 9 - protein, 12 aa, Artificial Sequence
  Linker
GGSSGGAGSGGG

SEQ ID NO: 10 - protein, 265 aa, Artificial Sequence
  Heavy Chain Fab <IGF-1>-GthCol mut
QVQLQQSGAELVRPGSSVKISCKASGYAFSNLWMNWVKQRPGQGLEWIGQIYPGDGDTNYYGDFKGKATLTADSSSSTAYMQLSRLTSEDSAVYFCARIGYYGMDYWGQGTSVTVSSGGSSGGAGSGGGGYNKGAIGIIPKEIRDKLVGKKFNSFDDFRKEFWKAVANSSYAKEFRSRNIARMLEGNAPIAPKAEHYGKLKSYILHAKQPIEKGGEVYNLDNLIITSPRMHQIILDPAYYFGKKGGGGYRYRQGGGSHHHHHHHH

SEQ ID NO: 11 - protein, 109 aa, Artificial Sequence
  Light Chain Fab <IGF-1>
DVVLTQTPLSLPVNIGDEASISCKSTKSLLSSDGLTYLDWYLQKPGQSPQVLIYLVSNRFSGVPDRFSGSGSGTDFTLKISRVEAEDLGVYYCFQSNYLPTFGAGTKLE

SEQ ID NO: 12 - protein, 219 aa, Artificial Sequence
  Heavy Chain Fab <IGF-1> -GthIM mut
QVQLQQSGAELVRPGSSVKISCKASGYAFSNLWMNWVKQRPGQGLEWIGQIYPGDGDTNYYGDFKGKATLTADSSSSTAYMQLSRLTSEDSAVYFCARIGYYGMDYWGQGTSVTVSSGGSSGGAGSGGGGENKLSKEELIELVKKIADPKLSDEEVSEYIDILEKNVPHPAPSDLIFWNDEELSPEEIVEIALNYKDRNGGGYRYRQGGGSHHHHHHHH

SEQ ID NO: 13 - protein, 137 aa, Artificial Sequence
  Gth colicin mut + aux
MGYNKGAIGIIPKEIRDKLVGKKFNSFDDFRKEFWKAVANSSYAKEFRSRNIARMLEGNAPIAPKAEHYGKLKSYILHAKQPIEKGGEVYNLDNLIITSPRMHQIILDPAYYFGKKGGGGYRYRQGGGSHHHHHHHH

SEQ ID NO: 14 - protein, 91 aa, Artificial Sequence
  Gth immunity mut. + aux
MGENKLSKEELIELVKKIADPKLSDEEVSEYIDILEKNVPHPAPSDLIFWNDEELSPEEIVEIALNYKDRNGGGYRYRQGGGSHHHHHHHH

SEQ ID NO: 15 - protein, 5 aa, Artificial Sequence
  transglutaminase peptide
YRYRQ

SEQ ID NO: 16 - protein, 115 aa, Artificial Sequence
  Gth colicin H77A
YNKGAIGIIPKEIRDKLVGKKFNSFDDFRKEFWKCVANSSYAKEFRSRNIARMLEGNAPIAPKAEHYGKLKSYILHAKQPIEKGGEVYNLDNLIITSPRMHQIILDPAYYFGKKG

SEQ ID NO: 17 - protein, 4 aa, Artificial Sequence
  repeating unit of poly(NANP)
NANP

SEQ ID NO: 18 - DNA, 411 bp, Artificial Sequence
  Gth colicin mut + aux encoding
atgggctacaacaaaggtgccattggcattattccgaaagaaattcgtgataaactggtgggcaaaaaattcaacagctttgatgatttccgcaaagagttttggaaagcagttgcaaatagcagctatgccaaagaatttcgtagccgtaatattgcacgtatgctggaaggtaatgcaccgattgcaccgaaagcagaacattatggtaaactgaaaagctatatcctgcatgccaaacagccgattgaaaaaggtggtgaagtttataatctggacaacctgattattaccagtccgcgtatgcatcagattattctggatccggcatattactttggtaaaaaaggcggtggtggttatcgttatcgtcaaggtggtggtagtcatcatcaccaccatcaccatcac

SEQ ID NO: 19 - DNA, 273 bp, Artificial Sequence
  GTH immunity mut + aux encoding
atgggcgagaacaaactgagcaaagaagaactgattgagctggtgaaaaaaatcgcagatccgaaactgagtgatgaagaagtgagcgagtatattgacatcctggaaaaaaatgttccgcatccggcaccgagcgatctgattttttggaacgatgaagaactgtcaccggaagaaattgttgaaattgccctgaactataaagatcgcaatggtggtggttatcgttatcgtcaaggtggtggcagtcatcatcaccaccatcaccatcac